European Patent Specification EP 4 493 207 B1, published March 11, 2026. Title: METHODS FOR PREVENTING AND TREATING BRAIN INFLAMMATION. Applicant: BIOXODES. The sequence listing filed with the application follows.

SEQUENCE LISTING (3 sequences)

SEQ ID NO: 1 - protein, 67 aa, Ixodes ricinus
ANHKGRGRPAKCKLPPDDGPCRARIPSYYFDRKTKTCKEFMYGGCEGNENNFENITTCQEECRAKKV

SEQ ID NO: 2 - protein, 67 aa, synthetic construct
ANHKGRGRPAKCKLPPDDGPCRARIPSYYFDRKTKTCKEFMYGGCEGNENNFEQITTCQEECRAKKV

SEQ ID NO: 3 - DNA, 204 bp, Ixodes ricinus
  source 1..204: mol_type = genomic DNA
gccaaccacaaaggtagagggcggcctgcgaagtgtaaacttcctccggacgacggaccatgcagagcacgaattccgagttactactttgatagaaaaaccaaaacgtgcaaggagtttatgtatggcggatgcgaaggaaacgaaaacaattttgaaaacataactacgtgccaagaggaatgcagagcaaaaaaagtctaa